European Patent Application EP 4 353 838 A1, published April 17, 2024. Title: METHOD FOR HEPATOCELLULAR CARCINOMA RISK STRATIFICATION. Applicant: ASSISTANCE PUBLIQUE HÔPITAUX DE PARIS. The sequence listing filed with the application follows.

SEQUENCE LISTING (4 sequences)

SEQ ID NO: 1 - DNA, 30 bp, synthetic construct
  source 1..30: mol_type = other DNA
gctctattggtgttttagtatttgggtgtt

SEQ ID NO: 2 - DNA, 33 bp, synthetic construct
  source 1..33: mol_type = other DNA
tgttccatcgtatatcaatatctttctgagact

SEQ ID NO: 3 - DNA, 19 bp, synthetic construct
  source 1..19: mol_type = other DNA
ctgtgctgtacttacttct

SEQ ID NO: 4 - DNA, 17 bp, synthetic construct
  source 1..17: mol_type = other DNA
tgctgtacttaacttct